European Patent Application EP 4 786 499 A1, published August 5, 2026. Title: 抗PD1-IL10融合蛋白及其应用. Applicant: 珠海菲鹏制药有限公司. The sequence listing filed with the application follows.

SEQUENCE LISTING (43 sequences)

SEQ ID NO: 1 - protein, 120 aa, synthetic construct
QVQLVQSGAEVKKPGASVKVSCKASGYTFTTYYMYWVRQAPGQGLEWMGGINPSNGGTNYAQKFQGRATMTVDTSTSTAYMELSSLRSEDTAVYYCTRRDSNYDGGFDYWGQGTTVTVSS

SEQ ID NO: 2 - protein, 111 aa, synthetic construct
DIQMTQSPSSLSASVGDRVTITCRASKSVSTSGYSYMHWYQQKPGKAPKLLIYLAYHLESGVPSRFSGSGSGTDFTLTISSLQPEDFATYYCQHSWELPITFGQGTKLEIK

SEQ ID NO: 3 - protein, 120 aa, synthetic construct
QVQLVQSGAEVKKPGASVKVSCKASGYTFTTYYMYWVRQAPGQGLEWMGGINPSNGGTNFNEKFKSRVTMTVDKSTSTAYMELSSLRSEDTAVYYCTRRDSNYDGGFDYWGQGTTVTVSS

SEQ ID NO: 4 - protein, 111 aa, synthetic construct
DIQLTQSPSSLSASVGDRATITCRASKSVSTSGYSYMHWYQQKPGKAPKLLIYLAYHLESGVPSRFSGSGSGTDFTLTISSVQPEDFATYYCQHSWELPITFGQGTKLEIK

SEQ ID NO: 5 - protein, 120 aa, synthetic construct
QVQLVQSGAEVKKPGASVKVSCKASGYTFTTYYMYWVRQAPGQGLEWIGGINPSNGGTNYAEKFKGRVTLTVDTSTSTAYMELSSLRSEDTAVYYCTRRDSNYDGGFDYWGQGTTVTVSS

SEQ ID NO: 6 - protein, 111 aa, synthetic construct; identical to SEQ ID NO: 2

SEQ ID NO: 7 - protein, 120 aa, synthetic construct
QVQLQQPGAELVKPGASVKLSCKASGYTFTTYYMYWVKQRPGQGLEWIGGINPSNGGTNFNEKFKSKATLTVDKSSSTAYMQLSSLTSEDSAVYYCTRRDSNYDGGFDYWGQGTTLTVSS

SEQ ID NO: 8 - protein, 111 aa, synthetic construct
DIVLTQSPASLAVSLGQRATISCRASKSVSTSGYSYMHWYQQKPGQPPKLLIYLAYHLESGVPARFSGSGSGTDFTLNIHPVEEEDAATYYCQHSWELPITFGSGTKLEIK

SEQ ID NO: 9 - protein, 5 aa, synthetic construct
TYYMY

SEQ ID NO: 10 - protein, 17 aa, synthetic construct
GINPSNGGTNYAQKFQG

SEQ ID NO: 11 - protein, 11 aa, synthetic construct
RDSNYDGGFDY

SEQ ID NO: 12 - protein, 15 aa, synthetic construct
RASKSVSTSGYSYMH

SEQ ID NO: 13 - protein, 7 aa, synthetic construct
LAYHLES

SEQ ID NO: 14 - protein, 9 aa, synthetic construct
QHSWELPIT

SEQ ID NO: 15 - protein, 17 aa, synthetic construct
GINPSNGGTNFNEKFKS

SEQ ID NO: 16 - protein, 17 aa, synthetic construct
GINPSNGGTNYAEKFKG

SEQ ID NO: 17 - protein, 450 aa, synthetic construct
QVQLVQSGAEVKKPGASVKVSCKASGYTFTTYYMYWVRQAPGQGLEWMGGINPSNGGTNYAQKFQGRATMTVDTSTSTAYMELSSLRSEDTAVYYCTRRDSNYDGGFDYWGQGTTVTVSSASTKGPSVFPLAPSSKSTSGGTAALGCLVKDYFPEPVTVSWNSGALTSGVHTFPAVLQSSGLYSLSSVVTVPSSSLGTQTYICNVNHKPSNTKVDKRVEPKSCDKTHTCPPCPAPEAAGGPSVFLFPPKPKDTLMISRTPEVTCVVVDVSHEDPEVKFNWYVDGVEVHNAKTKPREEQYNSTYRVVSVLTVLHQDWLNGKEYKCKVSNKALPAPIEKTISKAKGQPREPQVYTLPPSREEMTKNQVSLTCLVKGFYPSDIAVEWESNGQPENNYKTTPPVLDSDGSFFLYSKLTVDKSRWQQGNVFSCSVMHEALHNHYTQKSLSLSPGK

SEQ ID NO: 18 - protein, 218 aa, synthetic construct
DIQMTQSPSSLSASVGDRVTITCRASKSVSTSGYSYMHWYQQKPGKAPKLLIYLAYHLESGVPSRFSGSGSGTDFTLTISSLQPEDFATYYCQHSWELPITFGQGTKLEIKRTVAAPSVFIFPPSDEQLKSGTASVVCLLNNFYPREAKVQWKVDNALQSGNSQESVTEQDSKDSTYSLSSTLTLSKADYEKHKVYACEVTHQGLSSPVTKSFNRGEC

SEQ ID NO: 19 - protein, 330 aa, synthetic construct
ASTKGPSVFPLAPSSKSTSGGTAALGCLVKDYFPEPVTVSWNSGALTSGVHTFPAVLQSSGLYSLSSVVTVPSSSLGTQTYICNVNHKPSNTKVDKRVEPKSCDKTHTCPPCPAPEAAGGPSVFLFPPKPKDTLMISRTPEVTCVVVDVSHEDPEVKFNWYVDGVEVHNAKTKPREEQYNSTYRVVSVLTVLHQDWLNGKEYKCKVSNKALPAPIEKTISKAKGQPREPQVYTLPPSREEMTKNQVSLTCLVKGFYPSDIAVEWESNGQPENNYKTTPPVLDSDGSFFLYSKLTVDKSRWQQGNVFSCSVMHEALHNHYTQKSLSLSPGK

SEQ ID NO: 20 - protein, 107 aa, synthetic construct [sequence omitted]

SEQ ID NO: 21 - protein, 6 aa, synthetic construct
GGGSGG

SEQ ID NO: 22 - protein, 164 aa, synthetic construct
GQGTQSENSCTHFPGNLPNMLRDLRDAFSRVKTFFQMKDQLDNLLLKESLLEDFKGYLGCQALSEMIQFYLEEVMPQAENQDPDIKAHVNSLGENLKTLRLRLRRCHRFLPCENGGGSGGKSKAVEQVKNAFNKLQEKGIYKAMSEFDIFINYIEAYMTMKIRN

SEQ ID NO: 23 - protein, 160 aa, synthetic construct
SPGQGTQSENSCTHFPGNLPNMLRDLRDAFSRVKTFFQMKDQLDNLLLKESLLEDFKGYLGCQALSEMIQFYLEEVMPQAENQDPDIKAHVNSLGENLKTLRLRLRRCHRFLPCENKSKAVEQVKNAFNKLQEKGIYKAMSEFDIFINYIEAYMTMKIRN

SEQ ID NO: 24 - protein, 21 aa, synthetic construct
GGGGSGGGGSGGGGSGGGGSG

SEQ ID NO: 25 - protein, 403 aa, synthetic construct
DIQMTQSPSSLSASVGDRVTITCRASKSVSTSGYSYMHWYQQKPGKAPKLLIYLAYHLESGVPSRFSGSGSGTDFTLTISSLQPEDFATYYCQHSWELPITFGQGTKLEIKRTVAAPSVFIFPPSDEQLKSGTASVVCLLNNFYPREAKVQWKVDNALQSGNSQESVTEQDSKDSTYSLSSTLTLSKADYEKHKVYACEVTHQGLSSPVTKSFNRGECGGGGSGGGGSGGGGSGGGGSGGQGTQSENSCTHFPGNLPNMLRDLRDAFSRVKTFFQMKDQLDNLLLKESLLEDFKGYLGCQALSEMIQFYLEEVMPQAENQDPDIKAHVNSLGENLKTLRLRLRRCHRFLPCENGGGSGGKSKAVEQVKNAFNKLQEKGIYKAMSEFDIFINYIEAYMTMKIRN

SEQ ID NO: 26 - protein, 449 aa, synthetic construct
QVQLVESGGGVVQPGRSLRLSCAASGFTFSSYGMHWVRQAPGKGLEWVAAIWYDGSNKYYTDSVKGRFTISRDNSKNTLYLQMNSLRAEDTAVYYCARDLRGVMYFDLWGRGTLVTVSSASTKGPSVFPLAPSSKSTSGGTAALGCLVKDYFPEPVTVSWNSGALTSGVHTFPAVLQSSGLYSLSSVVTVPSSSLGTQTYICNVNHKPSNTKVDKRVEPKSCDKTHTCPPCPAPEAAGGPSVFLFPPKPKDTLMISRTPEVTCVVVDVSHEDPEVKFNWYVDGVEVHNAKTKPREEQYNSTYRVVSVLTVLHQDWLNGKEYKCKVSNKALPAPIEKTISKAKGQPREPQVYTLPPSREEMTKNQVSLTCLVKGFYPSDIAVEWESNGQPENNYKTTPPVLDSDGSFFLYSKLTVDKSRWQQGNVFSCSVMHEALHNHYTQKSLSLSPGK

SEQ ID NO: 27 - protein, 214 aa, synthetic construct
EIVLTQSPATLSLSPGERATLSCRASQSVSRYLAWYQQKPGQAPRLLIYDASNRATGIPARFSGSGSGTDFTLTISSLEPEDFAVYYCQLRNNWPLTFGGGTKVEIKRTVAAPSVFIFPPSDEQLKSGTASVVCLLNNFYPREAKVQWKVDNALQSGNSQESVTEQDSKDSTYSLSSTLTLSKADYEKHKVYACEVTHQGLSSPVTKSFNRGEC

SEQ ID NO: 28 - protein, 407 aa, synthetic construct
DKTHTCPPCPAPEAEGGPSVFLFPPKPKDTLMISRTPEVTCVVVDVSHEDPEVKFNWYVDGVEVHNAKTKPREEQYNSTYRVVSVLTVLHQDWLNGKEYKCKVSNKALPAPIEKTISKAKGQPREPQVYTLPPSREEMTKNQVSLTCLVKGFYPSDIAVEWESNGQPENNYKTTPPVLDSDGSFFLYSKLTVDKSRWQQGNVFSCSVMHEALHNHYTQKSLSLSPGKGGGGSGGGGSGGGGSGGGGSSPGQGTQSENSCTHFPGNLPNMLRDLRDAFSRVKTFFQMKDQLDNLLLKESLLEDFKGYLGCQALSEMIQFYLEEVMPQAENQDPDIKAHVNSLGENLKTLRLRLRRCHRFLPCENKSKAVEQVKNAFNKLQEKGIYKAMSEFDIFINYIEAYMTMKIRN

SEQ ID NO: 29 - protein, 626 aa, synthetic construct
QVQLKESGPGLVQPSQTLSLTCTVSGFSLTSYNVHWVRQPPGKGLEWMGGMRYNEDTSYNSALKSRLSISRDTSKNQVFLKMNSLQTDDTGTYYCTRDAVYGGYGGWFAYWGQGTLVTVSSAKTTPPSVYPLAPGSAAQTNSMVTLGCLVKGYFPEPVTVTWNSGSLSSGVHTFPAVLQSDLYTLSSSVTVPSSTWPSQTVTCNVAHPASSTKVDKKIVPRDCGCKPCICTVPEVSSVFIFPPKPKDVLTITLTPKVTCVVVAISKDDPEVQFSWFVDDVEVHTAQTKPREEQFNSTFRSVSELPIMHQDWLNGKEFKCRVNSAAFPAPIEKTISKTKGRPKAPQVYTIPPPKEQMAKDKVSLTCMITNFFPEDITVEWQWNGQPAENYKNTQPIMDTDGSYFVYSKLNVQKSNWEAGNTFTCSVLHEGLHNHHTEKSLSHSPGAGGGGSGGGGSGGGGSGGGGSGSPGQGTQSENSCTHFPGNLPNMLRDLRDAFSRVKTFFQMKDQLDNLLLKESLLEDFKGYLGCQALSEMIQFYLEEVMPQAENQDPDIKAHVNSLGENLKTLRLRLRRCHRFLPCENKSKAVEQVKNAFNKLQEKGIYKAMSEFDIFINYIEAYMTMKIRN

SEQ ID NO: 30 - protein, 216 aa, synthetic construct
DTVLTQSPALAVSLGQRVTISCKASETVSSSMYSYIHWYQQKPGQQPKLLIYRASNLESGVPARFSGSGSGTDFTLTIDPVEADDVATYFCQQSWNPWTFGGGTKLELKRADAAPTVSIFPPSSEQLTSGGASVVCFLNNFYPKDINVKWKIDGSERQNGVLNSWTDQDSKDSTYSMSSTLTLTKDEYERHNSYTCEATHKTSTSPIVKSFNRNEC

SEQ ID NO: 31 - protein, 407 aa, synthetic construct
DKTHTCPPCPAPEAAGGPSVFLFPPKPKDTLMISRTPEVTCVVVDVSQEDPEVQFNWYVDGVEVHNAKTKPREEQFNSTYRVVSVLTVLHQDWLNGKEYKCKVSNKGLPSSIEKTISKAKGQPREPQVYTLPPSQEEMTKNQVSLTCLVKGFYPSDIAVEWESNGQPENNYKTTPPVLDSDGSFFLYSRLTVDKSRWQEGNVFSCSVMHEALHNHYTQKSLSLSLGKGGGGSGGGGSGGGGSGGGGSSPGQGTQSENSCTHFPGNLPNMLRDLRDAFSRVKTFFQMKDQLDNLLLKESLLEDFKGYLGCQALSEMIQFYLEEVMPQAENQDPDIKAHVNSLGENLKTLRLRLRRCHRFLPCENKSKAVEQVKNAFNKLQEKGIYKAMSEFDIFINYIEAYMTMKIRN

SEQ ID NO: 32 - protein, 449 aa, synthetic construct; identical to SEQ ID NO: 26

SEQ ID NO: 33 - protein, 399 aa, synthetic construct
EIVLTQSPATLSLSPGERATLSCRASQSVSRYLAWYQQKPGQAPRLLIYDASNRATGIPARFSGSGSGTDFTLTISSLEPEDFAVYYCQLRNNWPLTFGGGTKVEIKRTVAAPSVFIFPPSDEQLKSGTASVVCLLNNFYPREAKVQWKVDNALQSGNSQESVTEQDSKDSTYSLSSTLTLSKADYEKHKVYACEVTHQGLSSPVTKSFNRGECGGGGSGGGGSGGGGSGGGGSGGQGTQSENSCTHFPGNLPNMLRDLRDAFSRVKTFFQMKDQLDNLLLKESLLEDFKGYLGCQALSEMIQFYLEEVMPQAENQDPDIKAHVNSLGENLKTLRLRLRRCHRFLPCENGGGSGGKSKAVEQVKNAFNKLQEKGIYKAMSEFDIFINYIEAYMTMKIRN

SEQ ID NO: 34 - protein, 630 aa, synthetic construct
QVQLVESGGGVVQPGRSLRLSCAASGFTFSSYGMHWVRQAPGKGLEWVAAIWYDGSNKYYTDSVKGRFTISRDNSKNTLYLQMNSLRAEDTAVYYCARDLRGVMYFDLWGRGTLVTVSSASTKGPSVFPLAPSSKSTSGGTAALGCLVKDYFPEPVTVSWNSGALTSGVHTFPAVLQSSGLYSLSSVVTVPSSSLGTQTYICNVNHKPSNTKVDKRVEPKSCDKTHTCPPCPAPEAAGGPSVFLFPPKPKDTLMISRTPEVTCVVVDVSHEDPEVKFNWYVDGVEVHNAKTKPREEQYNSTYRVVSVLTVLHQDWLNGKEYKCKVSNKALPAPIEKTISKAKGQPREPQVYTLPPSREEMTKNQVSLTCLVKGFYPSDIAVEWESNGQPENNYKTTPPVLDSDGSFFLYSKLTVDKSRWQQGNVFSCSVMHEALHNHYTQKSLSLSPGAGGGGSGGGGSGGGGSGGGGSGSPGQGTQSENSCTHFPGNLPNMLRDLRDAFSRVKTFFQMKDQLDNLLLKESLLEDFKGYLGCQALSEMIQFYLEEVMPQAENQDPDIKAHVNSLGENLKTLRLRLRRCHRFLPCENKSKAVEQVKNAFNKLQEKGIYKAMSEFDIFINYIEAYMTMKIRN

SEQ ID NO: 35 - protein, 214 aa, synthetic construct; identical to SEQ ID NO: 27

SEQ ID NO: 36 - protein, 447 aa, synthetic construct
QVQLVQSGVEVKKPGASVKVSCKASGYTFTNYYMYWVRQAPGQGLEWMGGINPSNGGTNFNEKFKNRVTLTTDSSTTTAYMELKSLQFDDTAVYYCARRDYRFDMGFDYWGQGTTVTVSSASTKGPSVFPLAPCSRSTSESTAALGCLVKDYFPEPVTVSWNSGALTSGVHTFPAVLQSSGLYSLSSVVTVPSSSLGTKTYTCNVDHKPSNTKVDKRVESKYGPPCPPCPAPEFLGGPSVFLFPPKPKDTLMISRTPEVTCVVVDVSQEDPEVQFNWYVDGVEVHNAKTKPREEQFNSTYRVVSVLTVLHQDWLNGKEYKCKVSNKGLPSSIEKTISKAKGQPREPQVYTLPPSQEEMTKNQVSLTCLVKGFYPSDIAVEWESNGQPENNYKTTPPVLDSDGSFFLYSRLTVDKSRWQEGNVFSCSVMHEALHNHYTQKSLSLSLGK

SEQ ID NO: 37 - protein, 218 aa, synthetic construct
EIVLTQSPATLSLSPGERATLSCRASKGVSTSGYSYLHWYQQKPGQAPRLLIYLASYLESGVPARFSGSGSGTDFTLTISSLEPEDFAVYYCQHSRDLPLTFGGGTKVEIKRTVAAPSVFIFPPSDEQLKSGTASVVCLLNNFYPREAKVQWKVDNALQSGNSQESVTEQDSKDSTYSLSSTLTLSKADYEKHKVYACEVTHQGLSSPVTKSFNRGEC

SEQ ID NO: 38 - protein, 451 aa, synthetic construct
QVQLKESGPGLVQPSQTLSLTCTVSGFSLTSYNVHWVRQPPGKGLEWMGGMRYNEDTSYNSALKSRLSISRDTSKNQVFLKMNSLQTDDTGTYYCTRDAVYGGYGGWFAYWGQGTLVTVSSASTKGPSVFPLAPSSKSTSGGTAALGCLVKDYFPEPVTVSWNSGALTSGVHTFPAVLQSSGLYSLSSVVTVPSSSLGTQTYICNVNHKPSNTKVDKRVEPKSCDKTHTCPPCPAPEAAGGPSVFLFPPKPKDTLMISRTPEVTCVVVDVSHEDPEVKFNWYVDGVEVHNAKTKPREEQYNSTYRVVSVLTVLHQDWLNGKEYKCKVSNKALPAPIEKTISKAKGQPREPQVYTLPPSREEMTKNQVSLTCLVKGFYPSDIAVEWESNGQPENNYKTTPPVLDSDGSFFLYSKLTVDKSRWQQGNVFSCSVMHEALHNHYTQKSLSLSPGK

SEQ ID NO: 39 - protein, 401 aa, synthetic construct
DTVLTQSPALAVSLGQRVTISCKASETVSSSMYSYIHWYQQKPGQQPKLLIYRASNLESGVPARFSGSGSGTDFTLTIDPVEADDVATYFCQQSWNPWTFGGGTKLELKRTVAAPSVFIFPPSDEQLKSGTASVVCLLNNFYPREAKVQWKVDNALQSGNSQESVTEQDSKDSTYSLSSTLTLSKADYEKHKVYACEVTHQGLSSPVTKSFNRGECGGGGSGGGGSGGGGSGGGGSGGQGTQSENSCTHFPGNLPNMLRDLRDAFSRVKTFFQMKDQLDNLLLKESLLEDFKGYLGCQALSEMIQFYLEEVMPQAENQDPDIKAHVNSLGENLKTLRLRLRRCHRFLPCENGGGSGGKSKAVEQVKNAFNKLQEKGIYKAMSEFDIFINYIEAYMTMKIRN

SEQ ID NO: 40 - protein, 451 aa, synthetic construct; identical to SEQ ID NO: 38

SEQ ID NO: 41 - protein, 216 aa, synthetic construct
DTVLTQSPALAVSLGQRVTISCKASETVSSSMYSYIHWYQQKPGQQPKLLIYRASNLESGVPARFSGSGSGTDFTLTIDPVEADDVATYFCQQSWNPWTFGGGTKLELKRTVAAPSVFIFPPSDEQLKSGTASVVCLLNNFYPREAKVQWKVDNALQSGNSQESVTEQDSKDSTYSLSSTLTLSKADYEKHKVYACEVTHQGLSSPVTKSFNRGEC

SEQ ID NO: 42 - protein, 450 aa, synthetic construct
QVQLVQSGAEVKKPGASVKVSCKASGYTFTTYYMYWVRQAPGQGLEWMGGINPSNGGTNYAQKFQGRATMTVDTSTSTAYMELSSLRSEDTAVYYCTRRDSNYDGGFDYWGQGTTVTVSSASTKGPSVFPLAPSSKSTSGGTAALGCLVKDYFPEPVTVSWNSGALTSGVHTFPAVLQSSGLYSLSSVVTVPSSSLGTQTYICNVNHKPSNTKVDKRVEPKSCDKTHTCPPCPAPELLGGPSVFLFPPKPKDTLMISRTPEVTCVVVDVSHEDPEVKFNWYVDGVEVHNAKTKPREEQYNSTYRVVSVLTVLHQDWLNGKEYKCKVSNKALPAPIEKTISKAKGQPREPQVYTLPPSREEMTKNQVSLTCLVKGFYPSDIAVEWESNGQPENNYKTTPPVLDSDGSFFLYSKLTVDKSRWQQGNVFSCSVMHEALHNHYTQKSLSLSPGK

SEQ ID NO: 43 - protein, 424 aa, synthetic construct
DIQMTQSPSSLSASVGDRVTITCRASKSVSTSGYSYMHWYQQKPGKAPKLLIYLAYHLESGVPSRFSGSGSGTDFTLTISSLQPEDFATYYCQHSWELPITFGQGTKLEIKRTVAAPSVFIFPPSDEQLKSGTASVVCLLNNFYPREAKVQWKVDNALQSGNSQESVTEQDSKDSTYSLSSTLTLSKADYEKHKVYACEVTHQGLSSPVTKSFNRGECGGGGSGGGGSGGGGSGGGGSGGGGGSGGGGSGGGGSGGGGSGGQGTQSENSCTHFPGNLPNMLRDLRDAFSRVKTFFQMKDQLDNLLLKESLLEDFKGYLGCQALSEMIQFYLEEVMPQAENQDPDIKAHVNSLGENLKTLRLRLRRCHRFLPCENGGGSGGKSKAVEQVKNAFNKLQEKGIYKAMSEFDIFINYIEAYMTMKIRN